European Patent Specification EP 3 802 871 B1, published September 24, 2025. Title: AMPLIFICATION METHOD. Applicant: Monoquant Pty Ltd. The sequence listing filed with the application follows.

SEQUENCE LISTING (19 sequences)

SEQ ID NO: 1 - DNA, 30 bp, Artificial Sequence
  AAMJ1b
ctttgctgagcacctgtccccaagtctgaa

SEQ ID NO: 2 - DNA, 23 bp, Artificial Sequence
  AAMJ2
aggccggctgcagaccccagata

SEQ ID NO: 3 - DNA, 26 bp, Artificial Sequence
  AAMJ3c
cccccggacattatctcccagctcca

SEQ ID NO: 4 - DNA, 34 bp, Artificial Sequence
  AAMJ4c
gcttatttccccccaaaaatgcagcaaaaccctt

SEQ ID NO: 5 - DNA, 32 bp, Artificial Sequence
  AAMJ5c
cctccaaaatgcctccaagactctgaccctga

SEQ ID NO: 6 - DNA, 31 bp, Artificial Sequence
  AAMJ6c
aggaaaccccacaggcagtagcagaaaacaa

SEQ ID NO: 7 - DNA, 31 bp, Artificial Sequence
  TCR1.1b
ttccctgtgacggatctgcaaaagaacctga

SEQ ID NO: 8 - DNA, 31 bp, Artificial Sequence
  TCR1.2b
ccctcctagagacccccagccttacctacaa

SEQ ID NO: 9 - DNA, 31 bp, Artificial Sequence
  TCR1.3b
caagttcccagctgtccagccttgacttact

SEQ ID NO: 10 - DNA, 39 bp, Artificial Sequence
  TCR1.4b
ccaggaactccgaccttatgatacactatcccgaaagaa

SEQ ID NO: 11 - DNA, 34 bp, Artificial Sequence
  TCR1.5b
atggccataccaccctgattctgcaacttaccta

SEQ ID NO: 12 - DNA, 28 bp, Artificial Sequence
  TCR1.6b
gagtcaagagtggagcccccatacctgt

SEQ ID NO: 13 - DNA, 27 bp, Artificial Sequence
  TCR2.1b
cacctggagcccccttcttacctagca

SEQ ID NO: 14 - DNA, 21 bp, Artificial Sequence
  TCR2.2b
cggagccccaaccgcctcctt

SEQ ID NO: 15 - DNA, 22 bp, Artificial Sequence
  TCR2.3b
ggagccccgcttaccgagcact

SEQ ID NO: 16 - DNA, 16 bp, Artificial Sequence
  TCR2.4b
ccggcggccccagctt

SEQ ID NO: 17 - DNA, 20 bp, Artificial Sequence
  TCR2.5b
gcgctcaccgagcaccagga

SEQ ID NO: 18 - DNA, 25 bp, Artificial Sequence
  TCR2.6b
cgcgaaaactcacccagcacggtca

SEQ ID NO: 19 - DNA, 23 bp, Artificial Sequence
  TCR2.7d
ggaaggtggggagacgcccgaat